European Patent Specification EP 4 352 258 B1, published July 29, 2026. Title: MATERIALS AND METHODS FOR MEASURING HPV CTDNA. Applicant: The Regents of the University of Michigan. The sequence listing filed with the application follows.

SEQUENCE LISTING (14 sequences)

SEQ ID NO: 1 - DNA, 24 bp, Artificial sequence
  Synthetic
cgaaaccggttagtataaaagcag

SEQ ID NO: 2 - DNA, 18 bp, Artificial sequence
  Synthetic
gtcgctcctgtgggtcct

SEQ ID NO: 3 - DNA, 34 bp, Artificial sequence
  Synthetic
cattttatgcaccaaaagagaactgcaatgtttc

SEQ ID NO: 4 - DNA, 77 bp, Artificial sequence
  Synthetic
cgaaaccggttagtataaaagcagacattttatgcaccaaaagagaactgcaatgtttcaggacccacaggagcgac

SEQ ID NO: 5 - DNA, 21 bp, Artificial sequence
  Synthetic
gaaccgaaccggttagtataa

SEQ ID NO: 6 - DNA, 19 bp, Artificial sequence
  Synthetic
ttgaaccgaaacggttagt

SEQ ID NO: 7 - DNA, 21 bp, Artificial sequence
  Synthetic
gttgaaccgaaaccggttagt

SEQ ID NO: 8 - DNA, 21 bp, Artificial sequence
  Synthetic
ttgaaccgaaaccggttagta

SEQ ID NO: 9 - DNA, 23 bp, Artificial sequence
  Synthetic
cgaaaccggttagtataaaagca

SEQ ID NO: 10 - DNA, 20 bp, Artificial sequence
  Synthetic
tgaaccgaaaccggttagta

SEQ ID NO: 11 - DNA, 23 bp, Artificial sequence
  Synthetic
ccgaaaccggttagtataaaagc

SEQ ID NO: 12 - DNA, 23 bp, Artificial sequence
  Synthetic
cgaaaccggttagtataaaagca

SEQ ID NO: 13 - DNA, 24 bp, Artificial sequence
  Synthetic
atgtatagttgtttgcagctctgt

SEQ ID NO: 14 - DNA, 19 bp, Artificial sequence
  Synthetic
ctttctgggtcgctcctgt